European Patent Specification EP 3 550 020 B1, published October 30, 2024. Title: IL6R BLOCK CAR-T TRANSGENIC VECTOR FOR ALLEVIATING CRS,PREPARATION METHOD THEREOF,AND APPLICATION OF THE SAME. Applicant: Shanghai Unicar-Therapy Bio-Medicine Technology Co., Ltd. The sequence listing filed with the application follows.

SEQUENCE LISTING (68 sequences)

SEQ ID NO: 1 - DNA, 861 bp, Artificial Sequence
  the sequence is synthetized
atgagtattcaacatttccgtgtcgcccttattcccttttttgcggcattttgccttcctgtttttgctcacccagaaacgctggtgaaagtaaaagatgctgaagatcagttgggtgcacgagtgggttacatcgaactggatctcaacagcggtaagatccttgagagttttcgccccgaagaacgttttccaatgatgagcacttttaaagttctgctatgtggcgcggtattatcccgtattgacgccgggcaagagcaactcggtcgccgcatacactattctcagaatgacttggttgagtactcaccagtcacagaaaagcatcttacggatggcatgacagtaagagaattatgcagtgctgccataaccatgagtgataacactgcggccaacttacttctgacaacgatcggaggaccgaaggagctaaccgcttttttgcacaacatgggggatcatgtaactcgccttgatcgttgggaaccggagctgaatgaagccataccaaacgacgagcgtgacaccacgatgcctgtagcaatggcaacaacgttgcgcaaactattaactggcgaactacttactctagcttcccggcaacaattaatagactggatggaggcggataaagttgcaggaccacttctgcgctcggcccttccggctggctggtttattgctgataaatctggagccggtgagcgtgggtctcgcggtatcattgcagcactggggccagatggtaagccctcccgtatcgtagttatctacacgacggggagtcaggcaactatggatgaacgaaatagacagatcgctgagataggtgcctcactgattaagcattggtaa

SEQ ID NO: 2 - DNA, 674 bp, Artificial Sequence
  the sequence is synthetized
cccgtagaaaagatcaaaggatcttcttgagatcctttttttctgcgcgtaatctgctgcttgcaaacaaaaaaaccaccgctaccagcggtggtttgtttgccggatcaagagctaccaactctttttccgaaggtaactggcttcagcagagcgcagataccaaatactgtccttctagtgtagccgtagttaggccaccacttcaagaactctgtagcaccgcctacatacctcgctctgctaatcctgttaccagtggctgctgccagtggcgataagtcgtgtcttaccgggttggactcaagacgatagttaccggataaggcgcagcggtcgggctgaacggggggttcgtgcacacagcccagcttggagcgaacgacctacaccgaactgagatacctacagcgtgagctatgagaaagcgccacgcttcccgaagggagaaaggcggacaggtatccggtaagcggcagggtcggaacaggagagcgcacgagggagcttccagggggaaacgcctggtatctttatagtcctgtcgggtttcgccacctctgacttgagcgtcgatttttgtgatgctcgtcaggggggcggagcctatggaaaaacgccagcaacgcggcctttttacggttcctggccttttgctggccttttgctcacat

SEQ ID NO: 3 - DNA, 147 bp, Artificial sequence
  the sequence is synthetized
atcccgcccctaactccgcccagttccgcccattctccgccccatggctgactaattttttttatttatgcagaggccgaggccgcctcggcctctgagctattccagaagtagtgaggaggcttttttggaggcctagacttttgc

SEQ ID NO: 4 - DNA, 228 bp, Artificial sequence
  the sequence is synthetized
gtagtcttatgcaatactcttgtagtcttgcaacatggtaacgatgagttagcaacatgccttacaaggagagaaaaagcaccgtgcatgccgattggtggaagtaaggtggtacgatcgtgccttattaggaaggcaacagacgggtctgacatggattggacgaaccactgaattgccgcattgcagagatattgtatttaagtgcctagctcgatacaataaacg

SEQ ID NO: 5 - DNA, 180 bp, Artificial sequence
  the sequence is synthetized
ggtctctctggttagaccagatctgagcctgggagctctctggctaactagggaacccactgcttaagcctcaataaagcttgccttgagtgcttcaagtagtgtgtgcccgtctgttgtgtgactctggtaactagagatccctcagacccttttagtcagtgtggaaaatctctagca

SEQ ID NO: 6 - DNA, 234 bp, Artificial sequence
  the sequence is synthetized
tgctagagattttccacactgactaaaagggtctgagggatctctagttaccagagtcacacaacagacgggcacacactacttgaagcactcaaggcaagctttattgaggcttaagcagtgggttccctagttagccagagagctcccaggctcagatctggtctaaccagagagacccagtacaagcaaaaagcagatcttattttcgttgggagtgaattagcccttcca

SEQ ID NO: 7 - DNA, 353 bp, Artificial sequence
  the sequence is synthetized
atgggtgcgagagcgtcagtattaagcgggggagaattagatcgcgatgggaaaaaattcggttaaggccagggggaaagaaaaaatataaattaaaacatatagtatgggcaagcagggagctagaacgattcgcagttaatcctggcctgttagaaacatcagaaggctgtagacaaatactgggacagctacaaccatcccttcagacaggatcagaagaacttagatcattatataatacagtagcaaccctctattgtgtgcatcaaaggatagagataaaagacaccaaggaagctttagacaagatagaggaagagcaaaacaaaagtaagaccaccgcacagcaa

SEQ ID NO: 8 - DNA, 233 bp, Artificial sequence
  the sequence is synthetized
aggagctttgttccttgggttcttgggagcagcaggaagcactatgggcgcagcctcaatgacgctgacggtacaggccagacaattattgtctggtatagtgcagcagcagaacaatttgctgagggctattgaggcgcaacagcatctgttgcaactcacagtctggggcatcaagcagctccaggcaagaatcctggctgtggaaagatacctaaaggatcaacagctcc

SEQ ID NO: 9 - DNA, 489 bp, Artificial sequence
  the sequence is synthetized
tggggatttggggttgctctggaaaactcatttgcaccactgctgtgccttggaatgctagttggagtaataaatctctggaacagattggaatcacacgacctggatggagtgggacagagaaattaacaattacacaagcttaatacactccttaattgaagaatcgcaaaaccagcaagaaaagaatgaacaagaattattggaattagataaatgggcaagtttgtggaattggtttaacataacaaattggctgtggtatataaaattattcataatgatagtaggaggcttggtaggtttaagaatagtttttgctgtactttctatagtgaatagagttaggcagggatattcaccattatcgtttcagacccacctcccaaccccgaggggacccgacaggcccgaaggaatagaagaagaaggtggagagagagacagagacagatccattcgattagtgaacggatctcgacggttaac

SEQ ID NO: 10 - DNA, 119 bp, Artificial sequence
  the sequence is synthetized
ttttaaaagaaaaggggggattggggggtacagtgcaggggaaagaatagtagacataatagcaacagacatacaaactaaagaattacaaaaacaaattacaaaaattcaaaatttta

SEQ ID NO: 11 - DNA, 592 bp, Artificial sequence
  the sequence is synthetized
aatcaacctctggattacaaaatttgtgaaagattgactggtattcttaactatgttgctccttttacgctatgtggatacgctgctttaatgcctttgtatcatgctattgcttcccgtatggctttcattttctcctccttgtataaatcctggttgctgtctctttatgaggagttgtggcccgttgtcaggcaacgtggcgtggtgtgcactgtgtttgctgacgcaacccccactggttggggcattgccaccacctgtcagctcctttccgggactttcgctttccccctccctattgccacggcggaactcatcgccgcctgccttgcccgctgctggacaggggctcggctgttgggcactgacaattccgtggtgttgtcggggaaatcatcgtcctttccttggctgctcgcctgtgttgccacctggattctgcgcgggacgtccttctgctacgtcccttcggccctcaatccagcggaccttccttcccgcggcctgctgccggctctgcggcctcttccgcgtcttcgccttcgccctcagacgagtcggatctccctttgggccgcctccccgcctg

SEQ ID NO: 12 - DNA, 1178 bp, Artificial sequence
  the sequence is synthetized
gctccggtgcccgtcagtgggcagagcgcacatcgcccacagtccccgagaagttggggggaggggtcggcaattgaaccggtgcctagagaaggtggcgcggggtaaactgggaaagtgatgtcgtgtactggctccgcctttttcccgagggtgggggagaaccgtatataagtgcagtagtcgccgtgaacgttctttttcgcaacgggtttgccgccagaacacaggtaagtgccgtgtgtggttcccgcgggcctggcctctttacgggttatggcccttgcgtgccttgaattacttccacctggctgcagtacgtgattcttgatcccgagcttcgggttggaagtgggtgggagagttcgaggccttgcgcttaaggagccccttcgcctcgtgcttgagttgaggcctggcctgggcgctggggccgccgcgtgcgaatctggtggcaccttcgcgcctgtctcgctgctttcgataagtctctagccatttaaaatttttgatgacctgctgcgacgctttttttctggcaagatagtcttgtaaatgcgggccaagatctgcacactggtatttcggtttttggggccgcgggcggcgacggggcccgtgcgtcccagcgcacatgttcggcgaggcggggcctgcgagcgcggccaccgagaatcggacgggggtagtctcaagctggccggcctgctctggtgcctggcctcgcgccgccgtgtatcgccccgccctgggcggcaaggctggcccggtcggcaccagttgcgtgagcggaaagatggccgcttcccggccctgctgcagggagctcaaaatggaggacgcggcgctcgggagagcgggcgggtgagtcacccacacaaaggaaaagggcctttccgtcctcagccgtcgcttcatgtgactccactgagtaccgggcgccgtccaggcacctcgattagttctcgagcttttggagtacgtcgtctttaggttggggggaggggttttatgcgatggagtttccccacactgagtgggtggagactgaagttaggccagcttggcacttgatgtaattctccttggaatttgccctttttgagtttggatcttggttcattctcaagcctcagacagtggttcaaagtttttttcttccatttcaggtgtcgtga

SEQ ID NO: 13 - DNA, 63 bp, Artificial sequence
  the sequence is synthetized
atggccttaccagtgaccgccttgctcctgccgctggccttgctgctccacgccgccaggccg

SEQ ID NO: 14 - DNA, 321 bp, Artificial sequence
  the sequence is synthetized
gacatccagatgacacagactacatcctccctgtctgcctctctgggagacagagtcaccatcagttgcagggcaagtcaggacattagtaaatatttaaattggtatcagcagaaaccagatggaactgttaaactcctgatctaccatacatcaagattacactcaggagtcccatcaaggttcagtggcagtgggtctggaacagattattctctcaccattagcaacctggagcaagaagatattgccacttacttttgccaacagggtaatacgcttccgtacacgttcggaggggggaccaagctggagatcaca

SEQ ID NO: 15 - DNA, 45 bp, Artificial sequence
  the sequence is synthetized
ggtggcggtggctcgggcggtggtgggtcgggtggcggcggatct

SEQ ID NO: 16 - DNA, 360 bp, Artificial sequence
  the sequence is synthetized
gaggtgaaactgcaggagtcaggacctggcctggtggcgccctcacagagcctgtccgtcacatgcactgtctcaggggtctcattacccgactatggtgtaagctggattcgccagcctccacgaaagggtctggagtggctgggagtaatatggggtagtgaaaccacatactataattcagctctcaaatccagactgaccatcatcaaggacaactccaagagccaagttttcttaaaaatgaacagtctgcaaactgatgacacagccatttactactgtgccaaacattattactacggtggtagctatgctatggactactggggccaaggaacctcagtcaccgtctcctca

SEQ ID NO: 17 - DNA, 141 bp, Artificial sequence
  the sequence is synthetized
accacgacgccagcgccgcgaccaccaacaccggcgcccaccatcgcgtcgcagcccctgtccctgcgcccagaggcgtgccggccagcggcggggggcgcagtgcacacgagggggctggacttcgcctgtgatatctac

SEQ ID NO: 18 - DNA, 66 bp, Artificial sequence
  the sequence is synthetized
atctgggcgcccttggccgggacttgtggggtccttctcctgtcactggttatcaccctttactgc

SEQ ID NO: 19 - DNA, 126 bp, Artificial sequence
  the sequence is synthetized
aaacggggcagaaagaaactcctgtatatattcaaacaaccatttatgagaccagtacaaactactcaagaggaagatggctgtagctgccgatttccagaagaagaagaaggaggatgtgaactg

SEQ ID NO: 20 - DNA, 336 bp, Artificial sequence
  the sequence is synthetized
agagtgaagttcagcaggagcgcagacgcccccgcgtacaagcagggccagaaccagctctataacgagctcaatctaggacgaagagaggagtacgatgttttggacaagagacgtggccgggaccctgagatggggggaaagccgagaaggaagaaccctcaggaaggcctgtacaatgaactgcagaaagataagatggcggaggcctacagtgagattgggatgaaaggcgagcgccggaggggcaaggggcacgatggcctttaccagggtctcagtacagccaccaaggacacctacgacgcccttcacatgcaggccctgccccctcgc

SEQ ID NO: 21 - DNA, 723 bp, Artificial sequence
  the sequence is synthetized
gacatccagatgacccagagcccaagcagcctgagcgccagcgtgggtgacagagtgaccatcacctgtagagccagccaggacatcagcagttacctgaattggtaccagcagaagccaggaaaggctccaaagctgctgatctactacacctccagactgcactctggtgtgccaagcagattcagcggtagcggtagcggtaccgacttcaccttcaccatcagcagcctccagccagaggacatcgctacctactactgccaacagggtaacacgcttccatacacgttcggccaagggaccaaggtggaaatcaaaggtggcggtggctcgggcggtggtgggtcgggtggcggcggatctcaggtccaactgcaggagagcggtccaggtcttgtgagacctagccagaccctgagcctgacctgcaccgtgtctggctactcaattaccagcgatcatgcctggagctgggttcgccagccacctggacgaggtcttgagtggattggatacattagttatagtggaatcacaacctataatccatctctcaaatccagagtgacaatgctgagagacaccagcaagaaccagttcagcctgagactcagcagcgtgacagccgccgacaccgcggtttattattgtgcaagatccctagctcggactacggctatggactactggggtcaaggcagcctcgtcacagtctcctca

SEQ ID NO: 22 - DNA, 747 bp, Artificial sequence
  the sequence is synthetized
gaaattgtgatgacccagagcccggcgaccctgagcgtgagcccgggcgaacgcgcgaccattacctgccgcgcgagccagggcattagcagctggctggcgtggtatcagcagaaaccgggccaggcgccgcgcctgctgatttatggcgcgagcacccgcgcgaccggcattccggcgcgctttagcggcagcggcagcggcaccgattttaccctgaccattagcagcctgcagccggaagattttgcggtgtattattgccagcagtatagcagctggccgccgtatacctttggccagggcaccaaactggaaattaaaggtggcggtggctcgggcggtggtgggtcgggtggcggcggatctgaagtgcagctggtggaaagcggcggcaacctggtgcagccgggccgcagcctgcgcctgagctgcgcggcgagcggctttatttttgatgattatgcgatgcattgggtgcgccaggcgccgggcaaaggcctggaatgggtgagcggcattagctggaacagcggcagcattggctatgcggatagcgtgaaaggccgctttaccattagccgcgataacgcgaaaaacagcctgtatctgcagatgaacagcctgcgcgcggaagataccgcgctgtattattgcgcgaaagatggcggcagcagctggctgccgtttgtgtattattatggcatggatgtgtggggccagggcaccaccgtgaccgtgagcagc

SEQ ID NO: 23 - DNA, 744 bp, Artificial sequence
  the sequence is synthetized
gatattcagatgacccagagcccgagcagcgtgagcgcgagcgtgggcgatcgcgtgaccctgagctgccgcgcgagccagagcattagcagcaactttgcgtggtatcagcagaaaccgggcaaagcgccgaaactgctgatttatggcgcgagcagcctggaaagcggcgtgccgagccgctttagcggcagcggcagcggcaccgattttaccctgaccattagcagcctgcagagcgaagattttgcgagctattattgccagcaggcgaacagctttccgtatacctttggccagggcaccaaactggaaattaaaggtggcggtggctcgggcggtggtgggtcgggtggcggcggatctgaagtgcagctggtggaaagcggcggcggcctggtgcagccgggccgcagcctgcgcctgagctgcgcggcgagcggctttatttttgatgattatgcgatgcattgggtgcgccaggcgccgggcaaaggcctggaatgggtgagcggcattagctggaacagcggcagcattggctatgcggatagcgtgaaaggccgctttaccattagccgcgataacgcgaaaaacagcctgtatctgcagatgaacagcctgcgcgcggaagataccgcgctgtattattgcgcgaaagatggcggcagcagctggctgccgtttgtgtattattatggcatggatgtgtggggccagggcaccaccgtgaccgtgagcagc

SEQ ID NO: 24 - DNA, 699 bp, Artificial sequence
  the sequence is synthetized
ttgttctggattcctgcttccatcagtgatgttgtgatgacccaaactgtcagtcttggagatcaagcttccatctcttgcagatctagtcagaaccttgtacacaacaatggaaacacctatttatattggttcctgcagaagtcaggccagtctccaaagctcctgatttatagggcttccatccgattttctggggtcccagacaggttcagtggcagtggatcagagacagatttcacactcaagatcagcagagtggaggcttatttctgctttcaaggtacacatgttccgtggacgttcggtggaggcaccaagctggaaatcaaaggtggcggtggctcgggcggtggtgggtcgggtggcggcggatctgaggtgctgctgcaacagtctggacctgagctggtgaagataccctgcaaggcttctggatacacattcactgactacaacatggactggatgaagcagagccatggaaagagccttgagtggattggagatattaatcctaagagtggtaattccatctacaaccagaagttcaagggcaaggccacactgactgtagacaagtcctccagcacagcctacatggagctccgcagcctgacatctgaggacactgcagtctatgactggtctgcctggtttgctttctggggccaagggactctggtctctgtctctgca

SEQ ID NO: 25 - DNA, 575 bp, Artificial sequence
  the sequence is synthetized
gcccctctccctcccccccccctaacgttactggccgaagccgcttggaataaggccggtgtgcgtttgtctatatgttattttccaccatattgccgtcttttggcaatgtgagggcccggaaacctggccctgtcttcttgacgagcattcctaggggtctttcccctctcgccaaaggaatgcaaggtctgttgaatgtcgtgaaggaagcagttcctctggaagcttcttgaagacaaacaacgtctgtagcgaccctttgcaggcagcggaaccccccacctggcgacaggtgcctctgcggccaaaagccacgtgtataagatacacctgcaaaggcggcacaaccccagtgccacgttgtgagttggatagttgtggaaagagtcaaatggctcacctcaagcgtattcaacaaggggctgaaggatgcccagaaggtaccccattgtatgggatctgatctggggcctcggtgcacatgctttacatgtgtttagtcgaggttaaaaaacgtctaggccccccgaaccacggggacgtggttttcctttgaaaaacacgatgataat

SEQ ID NO: 26 - DNA, 87 bp, Artificial sequence
  the sequence is synthetized
atgaactccttctccacaagcgccttcggtccagttgccttctccctggggctgctcctggtgttgcctgctgccttccctgcccca

SEQ ID NO: 27 - DNA, 696 bp, Artificial sequence
  the sequence is synthetized
gaaccgaaaagctgcgataaaacccatacctgcccgccgtgcccggcgccggaactgctgggcggcccgagcgtgtttctgtttccgccgaaaccgaaagataccctgatgattagccgcaccccggaagtgacctgcgtggtggtggatgtgagccatgaagatccggaagtgaaatttaactggtatgtggatggcgtggaagtgcataacgcgaaaaccaaaccgcgcgaagaacagtataacagcacctatcgcgtggtgagcgtgctgaccgtgctgcatcaggattggctgaacggcaaagaatataaatgcaaagtgagcaacaaagcgctgccggcgccgattgaaaaaaccattagcaaagcgaaaggccagccgcgcgaaccgcaggtgtataccctgccgccgagccgcgaagaaatgaccaaaaaccaggtgagcctgacctgcctggtgaaaggcttttatccgagcgatattgcggtggaatgggaaagcaacggccagccggaaaacaactataaaaccaccccgccggtgctggatagcgatggcagcttttttctgtatagcaaactgaccgtggataaaagccgctggcagcagggcaacgtgtttagctgcagcgtgatgcatgaagcgctgcataaccattatacccagaaaagcctgagcctgagcccgggcaaa

SEQ ID NO: 28 - DNA, 123 bp, Artificial sequence
  the sequence is synthetized
aggagtaagaggagcaggctcctgcacagtgactacatgaacatgactccccgccgccccgggcccacccgcaagcattaccagccctatgccccaccacgcgacttcgcagcctatcgctcc

SEQ ID NO: 29 - DNA, 36 bp, Artificial Sequence
  the sequence is synthetized
  misc_feature: Primer
attcaaaattttatcgatgctccggtgcccgtcagt

SEQ ID NO: 30 - DNA, 22 bp, Artificial sequence
  the sequence is synthetized
  misc_feature: Primer
tcacgacacctgaaatggaaga

SEQ ID NO: 31 - DNA, 42 bp, Artificial sequence
  the sequence is synthetized
  misc_feature: Primer
ggtgtcgtgaggatccgccaccatggccttaccagtgaccgc

SEQ ID NO: 32 - DNA, 31 bp, Artificial sequence
  the sequence is synthetized
  misc_feature: Primer
gtgtcatctggatgtccggcctggcggcgtg

SEQ ID NO: 33 - DNA, 41 bp, Artificial sequence
  the sequence is synthetized
  misc_feature: Primer
cacgccgccaggccggacatccagatgacacagactacatc

SEQ ID NO: 34 - DNA, 20 bp, Artificial sequence
  the sequence is synthetized
  misc_feature: Primer
tgtgatctccagcttggtcc

SEQ ID NO: 35 - DNA, 82 bp, Artificial sequence
  the sequence is synthetized
  misc_feature: Primer
caagctggagatcacaggtggcggtggctcgggcggtggtgggtcgggtggcggcggatctgaggtgaaactgcaggagtca

SEQ ID NO: 36 - DNA, 21 bp, Artificial sequence
  the sequence is synthetized
  misc_feature: Primer
tgaggagacggtgactgaggt

SEQ ID NO: 37 - DNA, 33 bp, Artificial sequence
  the sequence is synthetized
  misc_feature: Primer
agtcaccgtctcctcaaccacgacgccagcgcc

SEQ ID NO: 38 - DNA, 23 bp, Artificial sequence
  the sequence is synthetized
  misc_feature: Primer
gtagatatcacaggcgaagtcca

SEQ ID NO: 39 - DNA, 33 bp, Artificial sequence
  the sequence is synthetized
  misc_feature: Primer
cgcctgtgatatctacatctgggcgcccttggc

SEQ ID NO: 40 - DNA, 39 bp, Artificial sequence
  the sequence is synthetized
  misc_feature: Primer
tctttctgccccgtttgcagtaaagggtgataaccagtg

SEQ ID NO: 41 - DNA, 21 bp, Artificial sequence
  the sequence is synthetized
  misc_feature: Primer
aaacggggcagaaagaaactc

SEQ ID NO: 42 - DNA, 40 bp, Artificial sequence
  the sequence is synthetized
  misc_feature: Primer
tgctgaacttcactctcagttcacatcctccttcttcttc

SEQ ID NO: 43 - DNA, 22 bp, Artificial sequence
  the sequence is synthetized
  misc_feature: Primer
agagtgaagttcagcaggagcg

SEQ ID NO: 44 - DNA, 34 bp, Artificial sequence
  the sequence is synthetized
  misc_feature: Primer
ggagaggggcgtcgacttagcgagggggcagggc

SEQ ID NO: 45 - DNA, 34 bp, Artificial sequence
  the sequence is synthetized
  misc_feature: Primer
gccctgccccctcgctaagcccctctccctcccc

SEQ ID NO: 46 - DNA, 79 bp, Artificial sequence
  the sequence is synthetized
  misc_feature: Primer
ccagggagaaggcaactggaccgaaggcgcttgtggagaaggagttcatggtggcattatcatcgtgtttttcaaagga

SEQ ID NO: 47 - DNA, 74 bp, Artificial sequence
  the sequence is synthetized
  misc_feature: Primer
gttgccttctccctggggctgctcctggtgttgcctgctgccttccctgccccagacatccagatgacccagag

SEQ ID NO: 48 - DNA, 36 bp, Artificial sequence
  the sequence is synthetized
  misc_feature: Primer
gcagcttttcggttctgaggagactgtgacgaggct

SEQ ID NO: 49 - DNA, 74 bp, Artificial sequence
  the sequence is synthetized
  misc_feature: Primer
gttgccttctccctggggctgctcctggtgttgcctgctgccttccctgccccagaaattgtgatgacccagag

SEQ ID NO: 50 - DNA, 36 bp, Artificial sequence
  the sequence is synthetized
  misc_feature: Primer
gcagcttttcggttcgctgctcacggtcacggtggt

SEQ ID NO: 51 - DNA, 74 bp, Artificial sequence
  the sequence is synthetized
  misc_feature: Primer
gttgccttctccctggggctgctcctggtgttgcctgctgccttccctgccccagatattcagatgacccagag

SEQ ID NO: 52 - DNA, 36 bp, Artificial sequence; identical to SEQ ID NO: 50
  the sequence is synthetized
  misc_feature: Primer

SEQ ID NO: 53 - DNA, 76 bp, Artificial sequence
  the sequence is synthetized
  misc_feature: Primer
gttgccttctccctggggctgctcctggtgttgcctgctgccttccctgccccattgttctggattcctgcttcca

SEQ ID NO: 54 - DNA, 36 bp, Artificial sequence
  the sequence is synthetized
  misc_feature: Primer
gcagcttttcggttctgcagagacagagaccagagt

SEQ ID NO: 55 - DNA, 23 bp, Artificial sequence
  the sequence is synthetized
  misc_feature: Primer
gaaccgaaaagctgcgataaaac

SEQ ID NO: 56 - DNA, 38 bp, Artificial sequence
  the sequence is synthetized
  misc_feature: Primer
ctagcaatctagaggttatttgcccgggctcaggctca

SEQ ID NO: 57 - DNA, 21 bp, Artificial sequence
  the sequence is synthetized
  misc_feature: Primer
cctttccgggactttcgcttt

SEQ ID NO: 58 - DNA, 20 bp, Artificial sequence
  the sequence is synthetized
  misc_feature: Primer
gcagaatccaggtggcaaca

SEQ ID NO: 59 - DNA, 21 bp, Artificial sequence
  the sequence is synthetized
  misc_feature: Primer
catgtacgttgctatccaggc

SEQ ID NO: 60 - DNA, 21 bp, Artificial sequence
  the sequence is synthetized
  misc_feature: Primer
ctccttaatgtcacgcacgat

SEQ ID NO: 61 - DNA, 21 bp, Artificial sequence
  the sequence is synthetized
  misc_feature: Primer
gacttgtggggtccttctcct

SEQ ID NO: 62 - DNA, 21 bp, Artificial sequence
  the sequence is synthetized
  misc_feature: Primer
gcagctacagccatcttcctc

SEQ ID NO: 63 - DNA, 19 bp, Artificial sequence
  the sequence is synthetized
  misc_feature: Primer
ggattcaatgaggagactt

SEQ ID NO: 64 - DNA, 18 bp, Artificial sequence
  the sequence is synthetized
  misc_feature: Primer
atctgttctggaggtact

SEQ ID NO: 65 - DNA, 22 bp, Artificial sequence
  the sequence is synthetized
  misc_feature: Primer
gacattggaaatgtgaacatgt

SEQ ID NO: 66 - DNA, 19 bp, Artificial sequence
  the sequence is synthetized
  misc_feature: Primer
cacagctggggtttggtga

SEQ ID NO: 67 - DNA, 22 bp, Artificial sequence
  the sequence is synthetized
  misc_feature: Primer
gacattggaaatgtgaacatgt

SEQ ID NO: 68 - DNA, 19 bp, Artificial sequence
  the sequence is synthetized
  misc_feature: Primer
cacagctggggtttggtga